European Patent Application EP 4 481 044 A1, published December 25, 2024. Title: CELL SPECIFIC TRANSLATION OF RNA MOLECULES. Applicant: SRTD biotech GmbH. The sequence listing filed with the application follows.

SEQUENCE LISTING (4 sequences)

SEQ ID NO: 1 - RNA, 2308 nt, synthetic construct
  source 1..2308: mol_type = other RNA
tgatgtcggcctccacgctctggcgcagggccagctcattctcatacttgagcctgaagtcgtccgcagccagcctggcattgtcaatctccaggatgacccggttgttttcaatggtggcggtcaggatcttgtcccggagctcttcaatggtcttgtagtaggggctgtagtcccgctcagggctagctgggctctgcttcaggtgccagtcacggatcttcacctccaggtcagcgttggcctcctccagggcgcgcaccttctccaggtaggaagccaggcggtcgttgaggttctgcatggtgatcttctcattgccagtgaggaggccgccatcacaagcaccaaagtcaacaaagccaccagcaaaacccccaccaaagccacctccaaggccacctccatagccacctccaaggccacctccatagccacctccaaagccactaccagcccctccaccaaaaccacagctcacgccgcctccatagcccccagctgatcccccagacacaaaccgagttgaacaggtagagacaccacggcctcctcccagctggcaagagccacccccgaaaccacctccatagctggcagaggagctctgcaggcggaggctcatgaattcgttatgttatgaactgcttccttcacgacattcaacagaccttgttatgttattaaaagtcaggtcggatcaagccatagtacggaaaaaactatgctacctgtgagccccgtccaaggacgtgcggccgctaaaagaagtcaggccatcacaaatgccacagcttgagtaaactgtgcagcctgtagctccacctgagaaggtgtaagttatgttatggatcccccccctaacgttactggccgaagccgcttggaataaggccggtgtgcgtttgtctatatgttattttccaccatattgccgtcttttggcaatgtgagggcccggaaacctggccctgtcttcttgacgagcattcctaggggtctttcccctctcgccaaaggaatgcaaggtctgttgaatgtcgtgaaggaagcagttcctctggaagcttcttgaagacaaacaacgtctgtagcgaccctttgcaggcagcggaaccccccacctggcgacaggtgcctctgcggccaaaagccacgtgtataagatacacctgcaaaggcggcacaaccccagtgccacgttgtgagttggatagttgtggaaagagtcaaatggctctcctcaagcgtattcaacaaggggctgaaggatgcccagaaggtaccccattgtatgggatctgatctggggcctcggtgcacatgctttacatgtgtttagtcgaggttaaaaaacgtctaggccccccgaaccacggggacgtggttttcctttgaaaaacacgatgataatatggccacaaccatgtctagaatgattgagacagacagtggtgttgatgatgacatggcgtgtcataaaataccagtggaggccgacttcttgtatgcatactccacagcacctggttattattcttggcgaaattcaaaggatggctcctggttcatccagtcgctttgtgccatgctgaaacagtatgccgacaagcttgaatttatgcacattcttacccgggttaaccgaaaggtggcaacagaatttgagtccttttcctttgacgctacttttcatgcaaagaaacagattccatgtattgtttccatgctcacaaaagaactctatttttatcacgatgaagttgatgggggatcccccatggagaacactgaaaactcagtggattcaaaatccattaaaaatttggaaccaaagatcatacatggaagcgaatcaatggactctggaatatccctggacaacagttataaaatggattatcctgagatgggtttatgtataataattaataataagaattttcataagagcactggaatgacatctcggtctggtacagatgtcgatgcagcaaacctcagggaaacattcagaaacttgaaatatgaagtcaggaataaaaatgatcttacacgtgaagaaattgtggaattgatgcgtgatgtttctaaagaagatcacagcaaaaggagcagttttgtttgtgtgcttctgagccatggtgaagaaggaataatttttggaacaaatggacctgttgacctgaaaaaaataacaaactttttcagaggggatcgttgtagaagtctaactggaaaacccaaacttttcattattcaggcctgccgtggtacagaactggactgtggcattgagacagactga

SEQ ID NO: 2 - RNA, 2155 nt, synthetic construct
  source 1..2155: mol_type = other RNA
tgatgtcggcctccacgctctggcgcagggccagctcattctcatacttgagcctgaagtcgtccgcagccagcctggcattgtcaatctccaggatgacccggttgttttcaatggtggcggtcaggatcttgtcccggagctcttcaatggtcttgtagtaggggctgtagtcccgctcagggctagctgggctctgcttcaggtgccagtcacggatcttcacctccaggtcagcgttggcctcctccagggcgcgcaccttctccaggtaggaagccaggcggtcgttgaggttctgcatggtgatcttctcattgccagtgaggaggccgccatcacaagcaccaaagtcaacaaagccaccagcaaaacccccaccaaagccacctccaaggccacctccatagccacctccaaggccacctccatagccacctccaaagccactaccagcccctccaccaaaaccacagctcacgccgcctccatagcccccagctgatcccccagacacaaaccgagttgaacaggtagagacaccacggcctcctcccagctggcaagagccacccccgaaaccacctccatagctggcagaggagctctgcaggcggaggctcatgaattcgttatgttatgaactgcttccttcacgacattcaacagaccttgttatgttattaaaagtcaggtcggatcaagccatagtacggaaaaaactatgctacctgtgagccccgtccaaggacgtgcggccgctaaaagaagtcaggccatcacaaatgccacagcttgagtaaactgtgcagcctgtagctccacctgagaaggtgtaagttatgttatggatcccccccctaacgttactggccgaagccgcttggaataaggccggtgtgcgtttgtctatatgttattttccaccatattgccgtcttttggcaatgtgagggcccggaaacctggccctgtcttcttgacgagcattcctaggggtctttcccctctcgccaaaggaatgcaaggtctgttgaatgtcgtgaaggaagcagttcctctggaagcttcttgaagacaaacaacgtctgtagcgaccctttgcaggcagcggaaccccccacctggcgacaggtgcctctgcggccaaaagccacgtgtataagatacacctgcaaaggcggcacaaccccagtgccacgttgtgagttggatagttgtggaaagagtcaaatggctctcctcaagcgtattcaacaaggggctgaaggatgcccagaaggtaccccattgtatgggatctgatctggggcctcggtgcacatgctttacatgtgtttagtcgaggttaaaaaacgtctaggccccccgaaccacggggacgtggttttcctttgaaaaacacgatgataatatggccacaaccatgtctagaatggtgagcaagggcgaggagctgttcaccggggtggtgcccatcctggtcgagctggacggcgacgtaaacggccacaagttcagcgtgtccggcgagggcgagggcgatgccacctacggcaagctgaccctgaagttcatctgcaccaccggcaagctgcccgtgccctggcccaccctcgtgaccaccctgacctacggcgtgcagtgcttcagccgctaccccgaccacatgaagcagcacgacttcttcaagtccgccatgcccgaaggctacgtccaggagcgcaccatcttcttcaaggacgacggcaactacaagacccgcgccgaggtgaagttcgagggcgacaccctggtgaaccgcatcgagctgaagggcatcgacttcaaggaggacggcaacatcctggggcacaagctggagtacaactacaacagccacaacgtctatatcatggccgacaagcagaagaacggcatcaaggtgaacttcaagatccgccacaacatcgaggacggcagcgtgcagctcgccgaccactaccagcagaacacccccatcggcgacggccccgtgctgctgcccgacaaccactacctgagcacccagtccgccctgagcaaagaccccaacgagaagcgcgatcacatggtcctgctggagttcgtgaccgccgccgggatcactctcggcatggacgagctgtacaagtaa

SEQ ID NO: 3 - RNA, 60 nt, synthetic construct
  source 1..60: mol_type = other RNA
gggccgtccgggcaattgcccggacggccccccggcagcccgcaattgcgggctgccggg

SEQ ID NO: 4 - RNA, 68 nt, synthetic construct
  source 1..68: mol_type = other RNA
gcgcgccagggcgccaattggcgccctggcgcgcccgcgggtgggcgccaattggcgcccacccgcgg